European Patent Application EP 4 631 962 A1, published October 15, 2025. Title: Peptide for cartilage regeneration and uses thereof. Applicant: CAREGEN CO., LTD. The sequence listing filed with the application follows.

SEQUENCE LISTING (15 sequences)

SEQ ID NO: 1 - protein, 7 aa, synthetic construct
KRRRKRK

SEQ ID NO: 2 - DNA, 23 bp, synthetic construct
  source 1..23: mol_type = other DNA
ctatctggacgaagcagctggca

SEQ ID NO: 3 - DNA, 22 bp, synthetic construct
  source 1..22: mol_type = other DNA
atgggtgcaatgtcaatgatgg

SEQ ID NO: 4 - DNA, 20 bp, synthetic construct
  source 1..20: mol_type = other DNA
aactcagggcaggaggatgt

SEQ ID NO: 5 - DNA, 20 bp, synthetic construct
  source 1..20: mol_type = other DNA
tgtccttttggtcgtcgttc

SEQ ID NO: 6 - DNA, 20 bp, synthetic construct
  source 1..20: mol_type = other DNA
ccagcccgaacttgtaaaga

SEQ ID NO: 7 - DNA, 20 bp, synthetic construct
  source 1..20: mol_type = other DNA
tggacgcacaaccatcatac

SEQ ID NO: 8 - DNA, 20 bp, synthetic construct
  source 1..20: mol_type = other DNA
tgagtcctcaagcctcctgt

SEQ ID NO: 9 - DNA, 20 bp, synthetic construct
  source 1..20: mol_type = other DNA
gtgccagatcatcaccacac

SEQ ID NO: 10 - DNA, 20 bp, synthetic construct
  source 1..20: mol_type = other DNA
gcaggctatgagcagtgtga

SEQ ID NO: 11 - DNA, 20 bp, synthetic construct
  source 1..20: mol_type = other DNA
gcatacctcggaagcagaag

SEQ ID NO: 12 - DNA, 20 bp, synthetic construct
  source 1..20: mol_type = other DNA
accacagtccatgccatcac

SEQ ID NO: 13 - DNA, 20 bp, synthetic construct
  source 1..20: mol_type = other DNA
tccaccaccctgttgctgta

SEQ ID NO: 14 - DNA, 20 bp, synthetic construct
  source 1..20: mol_type = other DNA
gcggaggaagtcggtgaaga

SEQ ID NO: 15 - DNA, 20 bp, synthetic construct
  source 1..20: mol_type = other DNA
ccctctcgcttcaggtcagc